European Patent Application EP 4 643 882 A2, published November 5, 2025. Title: CAPSID INHIBITORS FOR THE PREVENTION OF HIV. Applicant: Gilead Sciences, Inc. Application EP. The sequence listing filed with the application follows.

SEQUENCE LISTING (3 sequences)

SEQ ID NO: 1 - DNA, 22 bp, synthetic construct
  misc_feature 1..22: note = synthetic oligonucleotides
  source 1..22: mol_type = other DNA
gtctgcgtcatctggtgcattc

SEQ ID NO: 2 - DNA, 29 bp, synthetic construct
  misc_feature 1..29: note = synthetic oligonucleotides
  source 1..29: mol_type = other DNA
cactaggtgtctctgcactatctgttttg

SEQ ID NO: 3 - DNA, 32 bp, synthetic construct
  misc_feature 1..32: note = synthetic oligonucleotides
  source 1..32: mol_type = other DNA
cttcctcagtgtgtttcactttctcttctgcg